European Patent Specification EP 3 699 198 B1, published March 26, 2025. Title: METHODS FOR TUMOR TREATMENT. Applicant: REGENERON PHARMACEUTICALS, INC. Application 62/080,716. The sequence listing filed with the application follows.

SEQUENCE LISTING (75 sequences)

SEQ ID NO: 1 - DNA, 382 bp, Artificial Sequence
  Synthetic
gaagtacagctggtggagtctgggggaggcttggtacagcctggcaggtccctgagactctcctgtgtagcctctggattcacctttaatgattatgccatgcactgggtccggcaagctccagggaagggcctggaatgggtctcagttattagttggaatagtgatagcataggctatgcggactctgtgaagggccgattcaccatctccagagacaacgccaagaactccctgtatctgcaaatgcacagtctgagagctgaggacacggccttgtattactgtgcaaaagataatcactatggttcggggagttattactactaccaatacggtatggacgtctggggccaagggaccacggtcaccgtctcctcag

SEQ ID NO: 2 - protein, 127 aa, Artificial Sequence
  Synthetic
EVQLVESGGGLVQPGRSLRLSCVASGFTFNDYAMHWVRQAPGKGLEWVSVISWNSDSIGYADSVKGRFTISRDNAKNSLYLQMHSLRAEDTALYYCAKDNHYGSGSYYYYQYGMDVWGQGTTVTVSS

SEQ ID NO: 3 - DNA, 24 bp, Artificial Sequence
  Synthetic
ggattcacctttaatgattatgcc

SEQ ID NO: 4 - protein, 8 aa, Artificial Sequence
  Synthetic
GFTFNDYA

SEQ ID NO: 5 - DNA, 24 bp, Artificial Sequence
  Synthetic
attagttggaatagtgatagcata

SEQ ID NO: 6 - protein, 8 aa, Artificial Sequence
  Synthetic
ISWNSDSI

SEQ ID NO: 7 - DNA, 60 bp, Artificial Sequence
  Synthetic
gcaaaagataatcactatggttcggggagttattactactaccaatacggtatggacgtc

SEQ ID NO: 8 - protein, 20 aa, Artificial Sequence
  Synthetic
AKDNHYGSGSYYYYQYGMDV

SEQ ID NO: 9 - DNA, 369 bp, Artificial Sequence
  Synthetic
gaagtgcagctggtggagtctgggggaggcttggtacagcctggcaggtccctgagactctcctgtgcagcctctggattcacctttgatgattataccatgcactgggtccggcaagctccagggaagggcctggagtgggtctcaggtattagttggaatagtggtagtataggctatgcggactctgtgaagggccgattcaccatctccagagacaacgccaagaagtccctgtatctgcaaatgaacagtctgagagctgaggacacggccttgtattactgtgcaaaagataatagtggctacggtcactactactacggaatggacgtctggggccaagggaccacggtcaccgtcgcctca

SEQ ID NO: 10 - protein, 123 aa, Artificial Sequence
  Synthetic
EVQLVESGGGLVQPGRSLRLSCAASGFTFDDYTMHWVRQAPGKGLEWVSGISWNSGSIGYADSVKGRFTISRDNAKKSLYLQMNSLRAEDTALYYCAKDNSGYGHYYYGMDVWGQGTTVTVAS

SEQ ID NO: 11 - DNA, 24 bp, Artificial Sequence
  Synthetic
ggattcacctttgatgattatacc

SEQ ID NO: 12 - protein, 8 aa, Artificial Sequence
  Synthetic
GFTFDDYT

SEQ ID NO: 13 - DNA, 24 bp, Artificial Sequence
  Synthetic
attagttggaatagtggtagtata

SEQ ID NO: 14 - protein, 8 aa, Artificial Sequence
  Synthetic
ISWNSGSI

SEQ ID NO: 15 - DNA, 48 bp, Artificial Sequence
  Synthetic
gcaaaagataatagtggctacggtcactactactacggaatggacgtc

SEQ ID NO: 16 - protein, 16 aa, Artificial Sequence
  Synthetic
AKDNSGYGHYYYGMDV

SEQ ID NO: 17 - DNA, 320 bp, Artificial Sequence
  Synthetic
gaaatagtgatgacgcagtctccagccaccctgtctgtgtctccaggggaaagagccaccctctcctgcagggccagtcagagtgttagcagcaacttagcctggtaccagcaaaaacctggccaggctcccaggctcctcatctatggtgcatccaccagggccactggtatcccagccaggttcagtggcagtgggtctgggacagagttcactctcaccatcagcagcctgcagtctgaagattttgcagtttattactgtcagcactatattaactggcctctcactttcggcggagggaccaaggtggagatcaa

SEQ ID NO: 18 - protein, 108 aa, Artificial Sequence
  Synthetic
EIVMTQSPATLSVSPGERATLSCRASQSVSSNLAWYQQKPGQAPRLLIYGASTRATGIPARFSGSGSGTEFTLTISSLQSEDFAVYYCQHYINWPLTFGGGTKVEIKR

SEQ ID NO: 19 - DNA, 18 bp, Artificial Sequence
  Synthetic
cagagtgttagcagcaac

SEQ ID NO: 20 - protein, 6 aa, Artificial Sequence
  Synthetic
QSVSSN

SEQ ID NO: 21 - DNA, 9 bp, Artificial Sequence
  Synthetic
ggtgcatcc

SEQ ID NO: 22 - protein, 3 aa, Artificial Sequence
  Synthetic
GAS

SEQ ID NO: 23 - DNA, 27 bp, Artificial Sequence
  Synthetic
cagcactatattaactggcctctcact

SEQ ID NO: 24 - protein, 9 aa, Artificial Sequence
  Synthetic
QHYINWPLT

SEQ ID NO: 25 - DNA, 981 bp, Artificial Sequence
  Synthetic
gccagcacaaaaggtcctagcgtttttccacttgccccatgttcaaggtcaacctccgaaagtaccgccgctcttggctgtctcgtaaaagattattttcccgaacctgtaactgtctcctggaactccggcgcactcacttccggcgtacataccttccccgctgtcctccaatcttccggtctctactccctgtcttctgttgtcactgttccatcatcctcactcggcacaaaaacatatacctgcaacgttgatcacaagccaagtaataccaaagttgataagcgcgtcgaatccaaatacggtcccccctgcccaccgtgcccagcaccacctgtggcaggaccatcagtcttcctgttccccccaaaacccaaggacactctcatgatctcccggacccctgaggtcacgtgcgtggtggtggacgtgagccaggaagaccccgaggtccagttcaactggtacgtggatggcgtggaggtgcataatgccaagacaaagccgcgggaggagcagttcaacagcacgtaccgtgtggtcagcgtcctcaccgtcctgcaccaggactggctgaacggcaaggagtacaagtgcaaggtctccaacaaaggcctcccgtcctccatcgagaaaaccatctccaaagccaaagggcagccccgagagccacaggtgtacaccctgcccccatcccaggaggagatgaccaagaaccaggtcagcctgacctgcctggtcaaaggcttctaccccagcgacatcgccgtggagtgggagagcaatgggcagccggagaacaactacaagaccacgcctcccgtgctggactccgacggctccttcttcctctacagcaggctcaccgtggacaagagcaggtggcaggaggggaatgtcttctcatgctccgtgatgcatgaggctctgcacaaccactacacacagaagtccctctccctgtctctgggtaaatga

SEQ ID NO: 26 - protein, 326 aa, Artificial Sequence
  Synthetic
ASTKGPSVFPLAPCSRSTSESTAALGCLVKDYFPEPVTVSWNSGALTSGVHTFPAVLQSSGLYSLSSVVTVPSSSLGTKTYTCNVDHKPSNTKVDKRVESKYGPPCPPCPAPPVAGPSVFLFPPKPKDTLMISRTPEVTCVVVDVSQEDPEVQFNWYVDGVEVHNAKTKPREEQFNSTYRVVSVLTVLHQDWLNGKEYKCKVSNKGLPSSIEKTISKAKGQPREPQVYTLPPSQEEMTKNQVSLTCLVKGFYPSDIAVEWESNGQPENNYKTTPPVLDSDGSFFLYSRLTVDKSRWQEGNVFSCSVMHEALHNHYTQKSLSLSLGK

SEQ ID NO: 27 - DNA, 981 bp, Artificial Sequence
  Synthetic
gccagcacaaaaggtcctagcgtttttccacttgccccatgttcaaggtcaacctccgaaagtaccgccgctcttggctgtctcgtaaaagattattttcccgaacctgtaactgtctcctggaactccggcgcactcacttccggcgtacataccttccccgctgtcctccaatcttccggtctctactccctgtcttctgttgtcactgttccatcatcctcactcggcacaaaaacatatacctgcaacgttgatcacaagccaagtaataccaaagttgataagcgcgtcgaatccaaatacggtcccccctgcccaccgtgcccagcaccacctgtggcaggaccatcagtcttcctgttccccccaaaacccaaggacactctcatgatctcccggacccctgaggtcacgtgcgtggtggtggacgtgagccaggaagaccccgaggtccagttcaactggtacgtggatggcgtggaggtgcataatgccaagacaaagccgcgggaggagcagttcaacagcacgtaccgtgtggtcagcgtcctcaccgtcctgcaccaggactggctgaacggcaaggagtacaagtgcaaggtctccaacaaaggcctcccgtcctccatcgagaaaaccatctccaaagccaaagggcagccccgagagccacaggtgtacaccctgcccccatcccaggaggagatgaccaagaaccaggtcagcctgacctgcctggtcaaaggcttctaccccagcgacatcgccgtggagtgggagagcaatgggcagccggagaacaactacaagaccacgcctcccgtgctggactccgacggctccttcttcctctacagcaggctcaccgtggacaagagcaggtggcaggaggggaatgtcttctcatgctccgtgatgcatgaggctctgcacaacagattcacacagaagtccctctccctgtctctgggtaaatga

SEQ ID NO: 28 - protein, 326 aa, Artificial Sequence
  Synthetic
ASTKGPSVFPLAPCSRSTSESTAALGCLVKDYFPEPVTVSWNSGALTSGVHTFPAVLQSSGLYSLSSVVTVPSSSLGTKTYTCNVDHKPSNTKVDKRVESKYGPPCPPCPAPPVAGPSVFLFPPKPKDTLMISRTPEVTCVVVDVSQEDPEVQFNWYVDGVEVHNAKTKPREEQFNSTYRVVSVLTVLHQDWLNGKEYKCKVSNKGLPSSIEKTISKAKGQPREPQVYTLPPSQEEMTKNQVSLTCLVKGFYPSDIAVEWESNGQPENNYKTTPPVLDSDGSFFLYSRLTVDKSRWQEGNVFSCSVMHEALHNRFTQKSLSLSLGK

SEQ ID NO: 29 - DNA, 990 bp, Artificial Sequence
  Synthetic
gcctccaccaagggcccatcggtcttccccctggcaccctcctccaagagcacctctgggggcacagcggccctgggctgcctggtcaaggactacttccccgaaccggtgacggtgtcgtggaactcaggcgccctgaccagcggcgtgcacaccttcccggctgtcctacagtcctcaggactctactccctcagcagcgtggtgaccgtgccctccagcagcttgggcacccagacctacatctgcaacgtgaatcacaagcccagcaacaccaaggtggacaagaaagttgagcccaaatcttgtgacaaaactcacacatgcccaccgtgcccagcaccacctgtggcaggaccatcagtcttcctgttccccccaaaacccaaggacactctcatgatctcccggacccctgaggtcacgtgcgtggtggtggacgtgagccaggaagaccccgaggtccagttcaactggtacgtggatggcgtggaggtgcataatgccaagacaaagccgcgggaggagcagttcaacagcacgtaccgtgtggtcagcgtcctcaccgtcctgcaccaggactggctgaacggcaaggagtacaagtgcaaggtctccaacaaaggcctcccgtcctccatcgagaaaaccatctccaaagccaaagggcagccccgagaaccacaggtgtacaccctgcccccatcccgggatgagctgaccaagaaccaggtcagcctgacctgcctggtcaaaggcttctatcccagcgacatcgccgtggagtgggagagcaatgggcagccggagaacaactacaagaccacgcctcccgtgctggactccgacggctccttcttcctctacagcaagctcaccgtggacaagagcaggtggcagcaggggaacgtcttctcatgctccgtgatgcatgaggctctgcacaaccactacacgcagaagtccctctccctgtctccgggtaaatga

SEQ ID NO: 30 - protein, 329 aa, Artificial Sequence
  Synthetic
ASTKGPSVFPLAPSSKSTSGGTAALGCLVKDYFPEPVTVSWNSGALTSGVHTFPAVLQSSGLYSLSSVVTVPSSSLGTQTYICNVNHKPSNTKVDKKVEPKSCDKTHTCPPCPAPPVAGPSVFLFPPKPKDTLMISRTPEVTCVVVDVSQEDPEVQFNWYVDGVEVHNAKTKPREEQFNSTYRVVSVLTVLHQDWLNGKEYKCKVSNKGLPSSIEKTISKAKGQPREPQVYTLPPSRDELTKNQVSLTCLVKGFYPSDIAVEWESNGQPENNYKTTPPVLDSDGSFFLYSKLTVDKSRWQQGNVFSCSVMHEALHNHYTQKSLSLSPGK

SEQ ID NO: 31 - DNA, 990 bp, Artificial Sequence
  Synthetic
gcctccaccaagggcccatcggtcttccccctggcaccctcctccaagagcacctctgggggcacagcggccctgggctgcctggtcaaggactacttccccgaaccggtgacggtgtcgtggaactcaggcgccctgaccagcggcgtgcacaccttcccggctgtcctacagtcctcaggactctactccctcagcagcgtggtgaccgtgccctccagcagcttgggcacccagacctacatctgcaacgtgaatcacaagcccagcaacaccaaggtggacaagaaagttgagcccaaatcttgtgacaaaactcacacatgcccaccgtgcccagcaccacctgtggcaggaccatcagtcttcctgttccccccaaaacccaaggacactctcatgatctcccggacccctgaggtcacgtgcgtggtggtggacgtgagccaggaagaccccgaggtccagttcaactggtacgtggatggcgtggaggtgcataatgccaagacaaagccgcgggaggagcagttcaacagcacgtaccgtgtggtcagcgtcctcaccgtcctgcaccaggactggctgaacggcaaggagtacaagtgcaaggtctccaacaaaggcctcccgtcctccatcgagaaaaccatctccaaagccaaagggcagccccgagaaccacaggtgtacaccctgcccccatcccgggatgagctgaccaagaaccaggtcagcctgacctgcctggtcaaaggcttctatcccagcgacatcgccgtggagtgggagagcaatgggcagccggagaacaactacaagaccacgcctcccgtgctggactccgacggctccttcttcctctacagcaagctcaccgtggacaagagcaggtggcagcaggggaacgtcttctcatgctccgtgatgcatgaggctctgcacaacagattcacgcagaagtccctctccctgtctccgggtaaatga

SEQ ID NO: 32 - protein, 329 aa, Artificial Sequence
  Synthetic
ASTKGPSVFPLAPSSKSTSGGTAALGCLVKDYFPEPVTVSWNSGALTSGVHTFPAVLQSSGLYSLSSVVTVPSSSLGTQTYICNVNHKPSNTKVDKKVEPKSCDKTHTCPPCPAPPVAGPSVFLFPPKPKDTLMISRTPEVTCVVVDVSQEDPEVQFNWYVDGVEVHNAKTKPREEQFNSTYRVVSVLTVLHQDWLNGKEYKCKVSNKGLPSSIEKTISKAKGQPREPQVYTLPPSRDELTKNQVSLTCLVKGFYPSDIAVEWESNGQPENNYKTTPPVLDSDGSFFLYSKLTVDKSRWQQGNVFSCSVMHEALHNRFTQKSLSLSPGK

SEQ ID NO: 33 - DNA, 981 bp, Artificial Sequence
  Synthetic
gccagcacaaaaggtcctagcgtttttccacttgccccatgttcaaggtcaacctccgaaagtaccgccgctcttggctgtctcgtaaaagattattttcccgaacctgtaactgtctcctggaactccggcgcactcacttccggcgtacataccttccccgctgtcctccaatcttccggtctctactccctgtcttctgttgtcactgttccatcatcctcactcggcacaaaaacatatacctgcaacgttgatcacaagccaagtaataccaaagttgataagcgcgtcgaatccaaatacggtcccccctgccccccatgtcccgctccacctgtggctggtccctctgttttcctttttccccctaaacccaaagataccctcatgatttccagaacccccgaggtcacctgcgtcgtcgttgatgtaagccaagaagatcccgaagtccagttcaattggtatgtagacggtgttgaagtccataatgcaaaaacaaaacccagagaggaacagtttaattcaacctatcgtgtcgttagcgtactcaccgttcttcatcaagactggctcaatggaaaagaatataaatgtaaagttagcaacaaaggtctgcccagttcaatcgaaaaaacaattagcaaagccaaaggccaacctcgcgaaccccaagtctataccttgcccccttctcaggaagaaatgaccaaaaaccaagtttcactcacatgcctcgtaaaaggattctatccatcagacattgcagtagaatgggaatctaacggccaacctgaaaataattacaaaaccactcctcctgtcctcgattctgacggctcttttttcctttactccagattgactgttgataaatcccgctggcaggaaggtaacgttttttcttgttctgtgatgcacgaagccctccataacagattcactcaaaaatctctttctctctccctgggcaaataa

SEQ ID NO: 34 - DNA, 645 bp, Artificial Sequence
  Synthetic
gaaatagtgatgacgcagtctccagccaccctgtctgtgtctccaggggaaagagccaccctctcctgcagggccagtcagagtgttagcagcaacttagcctggtaccagcagaaacctggccaggctcccaggctcctcatctatggtgcatccaccagggccactggtatcccagccaggttcagtggcagtgggtctgggacagagttcactctcaccatcagcagcctgcagtctgaagattttgcagtttattactgtcagcactatattaactggcctctcactttcggcggagggaccaaggtggagatcaaacgaactgtggctgcaccatctgtcttcatcttcccgccatctgatgagcagttgaaatctggaactgcctctgttgtgtgcctgctgaataacttctatcccagagaggccaaagtacagtggaaggtggataacgccctccaatcgggtaactcccaggagagtgtcacagagcaggacagcaaggacagcacctacagcctcagcagcaccctgacgctgagcaaagcagactacgagaaacacaaagtctacgcctgcgaagtcacccatcagggcctgagctcgcccgtcacaaagagcttcaacaggggagagtgttag

SEQ ID NO: 35 - protein, 214 aa, Artificial Sequence
  Synthetic
EIVMTQSPATLSVSPGERATLSCRASQSVSSNLAWYQQKPGQAPRLLIYGASTRATGIPARFSGSGSGTEFTLTISSLQSEDFAVYYCQHYINWPLTFGGGTKVEIKRTVAAPSVFIFPPSDEQLKSGTASVVCLLNNFYPREAKVQWKVDNALQSGNSQESVTEQDSKDSTYSLSSTLTLSKADYEKHKVYACEVTHQGLSSPVTKSFNRGEC

SEQ ID NO: 36 - DNA, 1362 bp, Artificial Sequence
  Synthetic
gaagtgcagctggtggagtctgggggaggcttggtacagcctggcaggtccctgagactctcctgtgtagcctctggattcacctttaatgattatgccatgcactgggtccggcaagctccagggaagggcctggaatgggtctcagttattagttggaatagtgatagcataggctatgcggactctgtgaagggccgattcaccatctccagagacaacgccaagaactccctgtatctgcaaatgcacagtctgagagctgaggacacggccttgtattactgtgcaaaagataatcactatggttcggggagttattactactaccaatacggtatggacgtctggggccaagggaccacggtcaccgtctcctcagccagcacaaaaggtcctagcgtttttccacttgccccatgttcaaggtcaacctccgaaagtaccgccgctcttggctgtctcgtaaaagattattttcccgaacctgtaactgtctcctggaactccggcgcactcacttccggcgtacataccttccccgctgtcctccaatcttccggtctctactccctgtcttctgttgtcactgttccatcatcctcactcggcacaaaaacatatacctgcaacgttgatcacaagccaagtaataccaaagttgataagcgcgtcgaatccaaatacggtcccccctgcccaccgtgcccagcaccacctgtggcaggaccatcagtcttcctgttccccccaaaacccaaggacactctcatgatctcccggacccctgaggtcacgtgcgtggtggtggacgtgagccaggaagaccccgaggtccagttcaactggtacgtggatggcgtggaggtgcataatgccaagacaaagccgcgggaggagcagttcaacagcacgtaccgtgtggtcagcgtcctcaccgtcctgcaccaggactggctgaacggcaaggagtacaagtgcaaggtctccaacaaaggcctcccgtcctccatcgagaaaaccatctccaaagccaaagggcagccccgagagccacaggtgtacaccctgcccccatcccaggaggagatgaccaagaaccaggtcagcctgacctgcctggtcaaaggcttctaccccagcgacatcgccgtggagtgggagagcaatgggcagccggagaacaactacaagaccacgcctcccgtgctggactccgacggctccttcttcctctacagcaggctcaccgtggacaagagcaggtggcaggaggggaatgtcttctcatgctccgtgatgcatgaggctctgcacaaccactacacacagaagtccctctccctgtctctgggtaaatga

SEQ ID NO: 37 - protein, 453 aa, Artificial Sequence
  Synthetic
EVQLVESGGGLVQPGRSLRLSCVASGFTFNDYAMHWVRQAPGKGLEWVSVISWNSDSIGYADSVKGRFTISRDNAKNSLYLQMHSLRAEDTALYYCAKDNHYGSGSYYYYQYGMDVWGQGTTVTVSSASTKGPSVFPLAPCSRSTSESTAALGCLVKDYFPEPVTVSWNSGALTSGVHTFPAVLQSSGLYSLSSVVTVPSSSLGTKTYTCNVDHKPSNTKVDKRVESKYGPPCPPCPAPPVAGPSVFLFPPKPKDTLMISRTPEVTCVVVDVSQEDPEVQFNWYVDGVEVHNAKTKPREEQFNSTYRVVSVLTVLHQDWLNGKEYKCKVSNKGLPSSIEKTISKAKGQPREPQVYTLPPSQEEMTKNQVSLTCLVKGFYPSDIAVEWESNGQPENNYKTTPPVLDSDGSFFLYSRLTVDKSRWQEGNVFSCSVMHEALHNHYTQKSLSLSLGK

SEQ ID NO: 38 - DNA, 1350 bp, Artificial Sequence
  Synthetic
gaagtgcagctggtggagtctgggggaggcttggtacagcctggcaggtccctgagactctcctgtgcagcctctggattcacctttgatgattataccatgcactgggtccggcaagctccagggaagggcctggagtgggtctcaggtattagttggaatagtggtagtataggctatgcggactctgtgaagggccgattcaccatctccagagacaacgccaagaagtccctgtatctgcaaatgaacagtctgagagctgaggacacggccttgtattactgtgcaaaagataatagtggctacggtcactactactacggaatggacgtctggggccaagggaccacggtcaccgtcgcctcagccagcacaaaaggtcctagcgtttttccacttgccccatgttcaaggtcaacctccgaaagtaccgccgctcttggctgtctcgtaaaagattattttcccgaacctgtaactgtctcctggaactccggcgcactcacttccggcgtacataccttccccgctgtcctccaatcttccggtctctactccctgtcttctgttgtcactgttccatcatcctcactcggcacaaaaacatatacctgcaacgttgatcacaagccaagtaataccaaagttgataagcgcgtcgaatccaaatacggtcccccctgcccaccgtgcccagcaccacctgtggcaggaccatcagtcttcctgttccccccaaaacccaaggacactctcatgatctcccggacccctgaggtcacgtgcgtggtggtggacgtgagccaggaagaccccgaggtccagttcaactggtacgtggatggcgtggaggtgcataatgccaagacaaagccgcgggaggagcagttcaacagcacgtaccgtgtggtcagcgtcctcaccgtcctgcaccaggactggctgaacggcaaggagtacaagtgcaaggtctccaacaaaggcctcccgtcctccatcgagaaaaccatctccaaagccaaagggcagccccgagagccacaggtgtacaccctgcccccatcccaggaggagatgaccaagaaccaggtcagcctgacctgcctggtcaaaggcttctaccccagcgacatcgccgtggagtgggagagcaatgggcagccggagaacaactacaagaccacgcctcccgtgctggactccgacggctccttcttcctctacagcaggctcaccgtggacaagagcaggtggcaggaggggaatgtcttctcatgctccgtgatgcatgaggctctgcacaacagattcacacagaagtccctctccctgtctctgggtaaatga

SEQ ID NO: 39 - DNA, 1350 bp, Artificial Sequence
  Synthetic
gaagtgcagctggtggagtctgggggaggcttggtacagcctggcaggtccctgagactctcctgtgcagcctctggattcacctttgatgattataccatgcactgggtccggcaagctccagggaagggcctggagtgggtctcaggtattagttggaatagtggtagtataggctatgcggactctgtgaagggccgattcaccatctccagagacaacgccaagaagtccctgtatctgcaaatgaacagtctgagagctgaggacacggccttgtattactgtgcaaaagataatagtggctacggtcactactactacggaatggacgtctggggccaagggaccacggtcaccgtcgcctcagccagcacaaaaggtcctagcgtttttccacttgccccatgttcaaggtcaacctccgaaagtaccgccgctcttggctgtctcgtaaaagattattttcccgaacctgtaactgtctcctggaactccggcgcactcacttccggcgtacataccttccccgctgtcctccaatcttccggtctctactccctgtcttctgttgtcactgttccatcatcctcactcggcacaaaaacatatacctgcaacgttgatcacaagccaagtaataccaaagttgataagcgcgtcgaatccaaatacggtcccccctgccccccatgtcccgctccacctgtggctggtccctctgttttcctttttccccctaaacccaaagataccctcatgatttccagaacccccgaggtcacctgcgtcgtcgttgatgtaagccaagaagatcccgaagtccagttcaattggtatgtagacggtgttgaagtccataatgcaaaaacaaaacccagagaggaacagtttaattcaacctatcgtgtcgttagcgtactcaccgttcttcatcaagactggctcaatggaaaagaatataaatgtaaagttagcaacaaaggtctgcccagttcaatcgaaaaaacaattagcaaagccaaaggccaacctcgcgaaccccaagtctataccttgcccccttctcaggaagaaatgaccaaaaaccaagtttcactcacatgcctcgtaaaaggattctatccatcagacattgcagtagaatgggaatctaacggccaacctgaaaataattacaaaaccactcctcctgtcctcgattctgacggctcttttttcctttactccagattgactgttgataaatcccgctggcaggaaggtaacgttttttcttgttctgtgatgcacgaagccctccataacagattcactcaaaaatctctttctctctccctgggcaaataa

SEQ ID NO: 40 - protein, 449 aa, Artificial Sequence
  Synthetic
EVQLVESGGGLVQPGRSLRLSCAASGFTFDDYTMHWVRQAPGKGLEWVSGISWNSGSIGYADSVKGRFTISRDNAKKSLYLQMNSLRAEDTALYYCAKDNSGYGHYYYGMDVWGQGTTVTVASASTKGPSVFPLAPCSRSTSESTAALGCLVKDYFPEPVTVSWNSGALTSGVHTFPAVLQSSGLYSLSSVVTVPSSSLGTKTYTCNVDHKPSNTKVDKRVESKYGPPCPPCPAPPVAGPSVFLFPPKPKDTLMISRTPEVTCVVVDVSQEDPEVQFNWYVDGVEVHNAKTKPREEQFNSTYRVVSVLTVLHQDWLNGKEYKCKVSNKGLPSSIEKTISKAKGQPREPQVYTLPPSQEEMTKNQVSLTCLVKGFYPSDIAVEWESNGQPENNYKTTPPVLDSDGSFFLYSRLTVDKSRWQEGNVFSCSVMHEALHNRFTQKSLSLSLGK

SEQ ID NO: 41 - DNA, 1371 bp, Artificial Sequence
  Synthetic
gaagtacagctggtggagtctgggggaggcttggtacagcctggcaggtccctgagactctcctgtgtagcctctggattcacctttaatgattatgccatgcactgggtccggcaagctccagggaagggcctggaatgggtctcagttattagttggaatagtgatagcataggctatgcggactctgtgaagggccgattcaccatctccagagacaacgccaagaactccctgtatctgcaaatgcacagtctgagagctgaggacacggccttgtattactgtgcaaaagataatcactatggttcggggagttattactactaccaatacggtatggacgtctggggccaagggaccacggtcaccgtctcctcagcctccaccaagggcccatcggtcttccccctggcaccctcctccaagagcacctctgggggcacagcggccctgggctgcctggtcaaggactacttccccgaaccggtgacggtgtcgtggaactcaggcgccctgaccagcggcgtgcacaccttcccggctgtcctacagtcctcaggactctactccctcagcagcgtggtgaccgtgccctccagcagcttgggcacccagacctacatctgcaacgtgaatcacaagcccagcaacaccaaggtggacaagaaagttgagcccaaatcttgtgacaaaactcacacatgcccaccgtgcccagcaccacctgtggcaggaccatcagtcttcctgttccccccaaaacccaaggacactctcatgatctcccggacccctgaggtcacgtgcgtggtggtggacgtgagccaggaagaccccgaggtccagttcaactggtacgtggatggcgtggaggtgcataatgccaagacaaagccgcgggaggagcagttcaacagcacgtaccgtgtggtcagcgtcctcaccgtcctgcaccaggactggctgaacggcaaggagtacaagtgcaaggtctccaacaaaggcctcccgtcctccatcgagaaaaccatctccaaagccaaagggcagccccgagaaccacaggtgtacaccctgcccccatcccgggatgagctgaccaagaaccaggtcagcctgacctgcctggtcaaaggcttctatcccagcgacatcgccgtggagtgggagagcaatgggcagccggagaacaactacaagaccacgcctcccgtgctggactccgacggctccttcttcctctacagcaagctcaccgtggacaagagcaggtggcagcaggggaacgtcttctcatgctccgtgatgcatgaggctctgcacaaccactacacgcagaagtccctctccctgtctccgggtaaatga

SEQ ID NO: 42 - protein, 456 aa, Artificial Sequence
  Synthetic
EVQLVESGGGLVQPGRSLRLSCVASGFTFNDYAMHWVRQAPGKGLEWVSVISWNSDSIGYADSVKGRFTISRDNAKNSLYLQMHSLRAEDTALYYCAKDNHYGSGSYYYYQYGMDVWGQGTTVTVSSASTKGPSVFPLAPSSKSTSGGTAALGCLVKDYFPEPVTVSWNSGALTSGVHTFPAVLQSSGLYSLSSVVTVPSSSLGTQTYICNVNHKPSNTKVDKKVEPKSCDKTHTCPPCPAPPVAGPSVFLFPPKPKDTLMISRTPEVTCVVVDVSQEDPEVQFNWYVDGVEVHNAKTKPREEQFNSTYRVVSVLTVLHQDWLNGKEYKCKVSNKGLPSSIEKTISKAKGQPREPQVYTLPPSRDELTKNQVSLTCLVKGFYPSDIAVEWESNGQPENNYKTTPPVLDSDGSFFLYSKLTVDKSRWQQGNVFSCSVMHEALHNHYTQKSLSLSPGK

SEQ ID NO: 43 - DNA, 1359 bp, Artificial Sequence
  Synthetic
gaagtgcagctggtggagtctgggggaggcttggtacagcctggcaggtccctgagactctcctgtgcagcctctggattcacctttgatgattataccatgcactgggtccggcaagctccagggaagggcctggagtgggtctcaggtattagttggaatagtggtagtataggctatgcggactctgtgaagggccgattcaccatctccagagacaacgccaagaagtccctgtatctgcaaatgaacagtctgagagctgaggacacggccttgtattactgtgcaaaagataatagtggctacggtcactactactacggaatggacgtctggggccaagggaccacggtcaccgtcgcctcagcctccaccaagggcccatcggtcttccccctggcaccctcctccaagagcacctctgggggcacagcggccctgggctgcctggtcaaggactacttccccgaaccggtgacggtgtcgtggaactcaggcgccctgaccagcggcgtgcacaccttcccggctgtcctacagtcctcaggactctactccctcagcagcgtggtgaccgtgccctccagcagcttgggcacccagacctacatctgcaacgtgaatcacaagcccagcaacaccaaggtggacaagaaagttgagcccaaatcttgtgacaaaactcacacatgcccaccgtgcccagcaccacctgtggcaggaccatcagtcttcctgttccccccaaaacccaaggacactctcatgatctcccggacccctgaggtcacgtgcgtggtggtggacgtgagccaggaagaccccgaggtccagttcaactggtacgtggatggcgtggaggtgcataatgccaagacaaagccgcgggaggagcagttcaacagcacgtaccgtgtggtcagcgtcctcaccgtcctgcaccaggactggctgaacggcaaggagtacaagtgcaaggtctccaacaaaggcctcccgtcctccatcgagaaaaccatctccaaagccaaagggcagccccgagaaccacaggtgtacaccctgcccccatcccgggatgagctgaccaagaaccaggtcagcctgacctgcctggtcaaaggcttctatcccagcgacatcgccgtggagtgggagagcaatgggcagccggagaacaactacaagaccacgcctcccgtgctggactccgacggctccttcttcctctacagcaagctcaccgtggacaagagcaggtggcagcaggggaacgtcttctcatgctccgtgatgcatgaggctctgcacaacagattcacgcagaagtccctctccctgtctccgggtaaatga

SEQ ID NO: 44 - protein, 452 aa, Artificial Sequence
  Synthetic
EVQLVESGGGLVQPGRSLRLSCAASGFTFDDYTMHWVRQAPGKGLEWVSGISWNSGSIGYADSVKGRFTISRDNAKKSLYLQMNSLRAEDTALYYCAKDNSGYGHYYYGMDVWGQGTTVTVASASTKGPSVFPLAPSSKSTSGGTAALGCLVKDYFPEPVTVSWNSGALTSGVHTFPAVLQSSGLYSLSSVVTVPSSSLGTQTYICNVNHKPSNTKVDKKVEPKSCDKTHTCPPCPAPPVAGPSVFLFPPKPKDTLMISRTPEVTCVVVDVSQEDPEVQFNWYVDGVEVHNAKTKPREEQFNSTYRVVSVLTVLHQDWLNGKEYKCKVSNKGLPSSIEKTISKAKGQPREPQVYTLPPSRDELTKNQVSLTCLVKGFYPSDIAVEWESNGQPENNYKTTPPVLDSDGSFFLYSKLTVDKSRWQQGNVFSCSVMHEALHNRFTQKSLSLSPGK

SEQ ID NO: 45 - protein, 330 aa, Artificial Sequence [sequence omitted]

SEQ ID NO: 46 - protein, 326 aa, Artificial Sequence
  Synthetic
ASTKGPSVFPLAPCSRSTSESTAALGCLVKDYFPEPVTVSWNSGALTSGVHTFPAVLQSSGLYSLSSVVTVPSSNFGTQTYTCNVDHKPSNTKVDKTVERKCCVECPPCPAPPVAGPSVFLFPPKPKDTLMISRTPEVTCVVVDVSHEDPEVQFNWYVDGVEVHNAKTKPREEQFNSTFRVVSVLTVVHQDWLNGKEYKCKVSNKGLPAPIEKTISKTKGQPREPQVYTLPPSREEMTKNQVSLTCLVKGFYPSDISVEWESNGQPENNYKTTPPMLDSDGSFFLYSKLTVDKSRWQQGNVFSCSVMHEALHNHYTQKSLSLSPGK

SEQ ID NO: 47 - protein, 327 aa, Artificial Sequence
  Synthetic
ASTKGPSVFPLAPCSRSTSESTAALGCLVKDYFPEPVTVSWNSGALTSGVHTFPAVLQSSGLYSLSSVVTVPSSSLGTKTYTCNVDHKPSNTKVDKRVESKYGPPCPSCPAPEFLGGPSVFLFPPKPKDTLMISRTPEVTCVVVDVSQEDPEVQFNWYVDGVEVHNAKTKPREEQFNSTYRVVSVLTVLHQDWLNGKEYKCKVSNKGLPSSIEKTISKAKGQPREPQVYTLPPSQEEMTKNQVSLTCLVKGFYPSDIAVEWESNGQPENNYKTTPPVLDSDGSFFLYSRLTVDKSRWQEGNVFSCSVMHEALHNHYTQKSLSLSLGK

SEQ ID NO: 48 - protein, 330 aa, Artificial Sequence
  Synthetic
ASTKGPSVFPLAPSSKSTSGGTAALGCLVKDYFPEPVTVSWNSGALTSGVHTFPAVLQSSGLYSLSSVVTVPSSSLGTQTYICNVNHKPSNTKVDKKVEPKSCDKTHTCPPCPAPELLGGPSVFLFPPKPKDTLMISRTPEVTCVVVDVSHEDPEVKFNWYVDGVEVHNAKTKPREEQYNSTYRVVSVLTVLHQDWLNGKEYKCKVSNKALPAPIEKTISKAKGQPREPQVYTLPPSRDELTKNQVSLTCLVKGFYPSDIAVEWESNGQPENNYKTTPPVLDSDGSFFLYSKLTVDKSRWQQGNVFSCSVMHEALHNRFTQKSLSLSPGK

SEQ ID NO: 49 - protein, 327 aa, Artificial Sequence
  Synthetic
ASTKGPSVFPLAPCSRSTSESTAALGCLVKDYFPEPVTVSWNSGALTSGVHTFPAVLQSSGLYSLSSVVTVPSSSLGTKTYTCNVDHKPSNTKVDKRVESKYGPPCPSCPAPEFLGGPSVFLFPPKPKDTLMISRTPEVTCVVVDVSQEDPEVQFNWYVDGVEVHNAKTKPREEQFNSTYRVVSVLTVLHQDWLNGKEYKCKVSNKGLPSSIEKTISKAKGQPREPQVYTLPPSQEEMTKNQVSLTCLVKGFYPSDIAVEWESNGQPENNYKTTPPVLDSDGSFFLYSRLTVDKSRWQEGNVFSCSVMHEALHNRFTQKSLSLSLGK

SEQ ID NO: 50 - protein, 12 aa, Artificial Sequence
  Synthetic
EPKSCDKTHTCP

SEQ ID NO: 51 - protein, 9 aa, Artificial Sequence
  Synthetic
ESKYGPPCP

SEQ ID NO: 52 - protein, 8 aa, Artificial Sequence
  Synthetic
PCPAPPVA

SEQ ID NO: 53 - protein, 20 aa, Artificial Sequence
  Synthetic
EPKSCDKTHTCPPCPAPPVA

SEQ ID NO: 54 - protein, 17 aa, Artificial Sequence
  Synthetic
ESKYGPPCPPCPAPPVA

SEQ ID NO: 55 - protein, 104 aa, Artificial Sequence
  Synthetic
GPSVFLFPPKPKDTLMISRTPEVTCVVVDVSQEDPEVQFNWYVDGVEVHNAKTKPREEQFNSTYRVVSVLTVLHQDWLNGKEYKCKVSNKGLPSSIEKTISKAK

SEQ ID NO: 56 - protein, 107 aa, Artificial Sequence
  Synthetic
GQPREPQVYTLPPSRDELTKNQVSLTCLVKGFYPSDIAVEWESNGQPENNYKTTPPVLDSDGSFFLYSKLTVDKSRWQQGNVFSCSVMHEALHNHYTQKSLSLSPGK

SEQ ID NO: 57 - protein, 107 aa, Artificial Sequence
  Synthetic
GQPREPQVYTLPPSRDELTKNQVSLTCLVKGFYPSDIAVEWESNGQPENNYKTTPPVLDSDGSFFLYSKLTVDKSRWQQGNVFSCSVMHEALHNRFTQKSLSLSPGK

SEQ ID NO: 58 - protein, 107 aa, Artificial Sequence
  Synthetic
GQPREPQVYTLPPSQEEMTKNQVSLTCLVKGFYPSDIAVEWESNGQPENNYKTTPPVLDSDGSFFLYSRLTVDKSRWQEGNVFSCSVMHEALHNHYTQKSLSLSLGK

SEQ ID NO: 59 - protein, 107 aa, Artificial Sequence
  Synthetic
GQPREPQVYTLPPSQEEMTKNQVSLTCLVKGFYPSDIAVEWESNGQPENNYKTTPPVLDSDGSFFLYSRLTVDKSRWQEGNVFSCSVMHEALHNRFTQKSLSLSLGK

SEQ ID NO: 60 - protein, 98 aa, Artificial Sequence
  Synthetic
ASTKGPSVFPLAPSSKSTSGGTAALGCLVKDYFPEPVTVSWNSGALTSGVHTFPAVLQSSGLYSLSSVVTVPSSSLGTQTYICNVNHKPSNTKVDKKV

SEQ ID NO: 61 - protein, 98 aa, Artificial Sequence
  Synthetic
ASTKGPSVFPLAPCSRSTSESTAALGCLVKDYFPEPVTVSWNSGALTSGVHTFPAVLQSSGLYSLSSVVTVPSSSLGTKTYTCNVDHKPSNTKVDKRV

SEQ ID NO: 62 - protein, 106 aa, Artificial Sequence
  Synthetic
TVAAPSVFIFPPSDEQLKSGTASVVCLLNNFYPREAKVQWKVDNALQSGNSQESVTEQDSKDSTYSLSSTLTLSKADYEKHKVYACEVTHQGLSSPVTKSFNRGEC

SEQ ID NO: 63 - DNA, 60 bp, Artificial Sequence
  Synthetic
ttcgcgcagcttaggtttatgccaggggggacgggtggcacgggtcgtggtggacaccgt

SEQ ID NO: 64 - DNA, 40 bp, Artificial Sequence
  Synthetic
aagcttatactcgagctctagattgggaacccgggtctct

SEQ ID NO: 65 - DNA, 58 bp, Artificial Sequence
  Synthetic
cccaccgtgcccagcaccacctgtggcaggaccatcagtcttcctgttccccccaaaa

SEQ ID NO: 66 - DNA, 44 bp, Artificial Sequence
  Synthetic
tgtgtcttcagggagagggacagagacccatttactcgccggcg

SEQ ID NO: 67 - DNA, 60 bp, Artificial Sequence
  Synthetic
ctcgggtttagaacactgttttgagtgtgtacgggtggcacgggtcgtggtggacaccgt

SEQ ID NO: 68 - DNA, 51 bp, Artificial Sequence
  Synthetic
aaatcttgtgacaaaactcacacatgcccaccgtgcccagcaccacctgtg

SEQ ID NO: 69 - DNA, 54 bp, Artificial Sequence
  Synthetic
gagaaaaccatctccaaagccaaagggcagccccgagaaccacaggtgtacacc

SEQ ID NO: 70 - DNA, 54 bp, Artificial Sequence
  Synthetic
ctcttttggtagaggtttcggtttcccgtcggggctcttggtgtccacatgtgg

SEQ ID NO: 71 - DNA, 39 bp, Artificial Sequence
  Synthetic
cttcagggagagggacagaggcccatttactcgccggcg

SEQ ID NO: 72 - DNA, 20 bp, Artificial Sequence
  Synthetic
gctgacagactaacagactg

SEQ ID NO: 73 - DNA, 26 bp, Artificial Sequence
  Synthetic
atacattatacgaagttataccggta

SEQ ID NO: 74 - protein, 105 aa, Artificial Sequence [sequence omitted]

SEQ ID NO: 75 - protein, 108 aa, Artificial Sequence
  Synthetic
AEIVMTQSPATLSVSPGERATLSCRASQSVSSNLAWYQQKPGQAPRLLIYGASTRATGIPARFSGSGSGTEFTLTISSLQSEDFAVYYCQHYINWPLTFGGGTKVEIK